European Patent Application EP 4 516 908 A1, published March 5, 2025. Title: PROTEIN HAVING NAMPT ACTIVITY AND METHOD FOR PRODUCING NMN. Applicant: KYOWA HAKKO BIO CO., LTD. The sequence listing filed with the application follows.

SEQUENCE LISTING (27 sequences)

SEQ ID NO: 1 - DNA, 1473 bp, Bisgaardia hudsonensis
  source 1..1473: mol_type = genomic DNA
atgtttaatttacaacattctacagccattcctaccttaatgtgtgatttttataaagtatcacaccgtgagcaatatccagaaggttcgcaagttatttatagtacgtttacaccacgtagtaacaaacgtgctccacacttggatagagcggtatcttttggttttcaagcatttatcaaaaaataccttatacattattttaatcaaaatttcttttctcgccctttagatgaagttttacaggaatattcagcgttcattaagcgtacattaggtacggaagatggtgggaaacatattgcggaactgcataaattgggttatttaccgattaaaattaaaactattcctgagggaaaatcggtagcaattaaagttcctatgctgactattgaaaatacgcataatgacttcttttggttgactaattacttagaaaccttgattaatatgtctttatggcaacctattgtatcagcaagtgttgcgagagtttatcgtaagacattaatgagttttgcagaaaaaacttgtgataatcaagagcatataccttttcaagcccatgatttttcaatgcgaggtatgagttctttagaaacagcggaaacatcaggtgctgggcatttaactgcttttttaggtacggatacgatacctgctatttcttttattgaaggctattatggttctaaaaatttaattggcacgtcaattccagcaacagaacattctgtgatgagtgctcacggtattgatgagttaccgacttttcgttatttaatgaaaaaatacccaaattctatgttgtctatcgtttcagatactacggatttctggcataacataacggttaatttacctattttaagagatgagattatggctcgtccagatcacgcaaaaatcattattcgtcctgatagtggcgatagctataagattatttgcggtgataaggacgctaaaactgaacatgaacaaaaaggtttaattgaatgtttgtgggatacttttggtggtacagttaatcgtaaagggtataaagttcttgattgccatattggtgctatttatggcgatggtgttaattatgaaaaaatgacaaggattttagagggcttaacggaaaaaggatttgcatcaagtaatcttgtttttggcgttgggtcattaacttatcaaaatcatactcgagatactttaggttttgccgttaaagcaacctcaattattatcaacaatgaagaaaaggcgatttttaaaaatcctaaaactgatgatggtttaaaaaaatctcaaaaaggtcgggtaaaagttctttctcttgatcactatattgatggattatcaacaaaagatgatttctctgatgatgtattagaaactatttttgaaaatggaaaattattaaaagagattaactttgattcagtgagagaaaatatgttatcagaattgaatggataa

SEQ ID NO: 2 - DNA, 1473 bp, Bisgaardia hudsonensis
  source 1..1473: mol_type = other DNA
atgtttaacctgcagcatagcacagccattccgaccttaatgtgcgatttctacaaagtctctcatcgcgaacagtatccggaaggatcgcaggtgatttatagcacctttactccgagatcaaacaagcgtgcacctcatttagaccgtgcggtatcctttgggtttcaagcgttcattaaaaagtatctgatccattacttcaatcagaacttcttctcacgtccgttagatgaagttctgcaggaatattcggcattcataaaacgcaccttagggactgaagatggcggcaaacatatcgcggaattacacaaactgggttatttgcctatcaagatcaagaccatccccgaagggaagtctgttgcgattaaagttccgatgctaaccattgagaatacccacaacgacttcttttggctcaccaactatttggaaacgctgataaatatgtcactgtggcaaccgattgtttctgccagtgtggctcgggtgtaccgcaaaaccctgatgagctttgcggaaaaaacgtgcgataatcaggagcatattccgtttcaagctcacgatttttcgatgcgtggtatgtctagtcttgaaactgcggagacaagtggtgcaggacatctgacggcttttctgggcacagataccattccggctattagcttcattgagggctactatggctctaaaaaccttatcggaacatcgattccggccaccgaacacagcgtaatgtcagcacatggtattgacgaactgccgactttccgctatctgatgaaaaaataccccaattcgatgctcagcattgtgagcgacaccacggacttttggcacaacattaccgtgaacttgccaatactccgtgacgaaattatggcacgaccagatcacgcgaaaatcattatccgccctgattcgggtgattcctacaaaatcatctgtggggacaaagatgcgaaaacagagcacgaacagaaaggtcttatcgagtgtctgtgggacacctttggcggtactgtcaatcgtaaagggtataaggtcctcgattgccatattggtgccatttatggcgatggtgtgaattacgaaaaaatgacccgcattctggaaggtctgacggaaaagggctttgcctccagcaatctggtctttggtgttggctcattgacctatcagaaccatacgcgggatacgctaggcttcgcggtaaaagccacgtccatcatcatcaacaatgaagagaaagccatctttaaaaacccaaaaaccgatgatggcctgaaaaagagtcaaaaaggccgcgttaaagtcctgagcctggatcactacattgacggcttatccacgaaagacgacttcagcgatgatgtgttggaaactatcttcgaaaatggaaaacttctgaaagagatcaactttgatagtgtgcgtgagaacatgctgagtgaactgaatggctaa

SEQ ID NO: 3 - protein, 490 aa, Bisgaardia hudsonensis
MFNLQHSTAIPTLMCDFYKVSHREQYPEGSQVIYSTFTPRSNKRAPHLDRAVSFGFQAFIKKYLIHYFNQNFFSRPLDEVLQEYSAFIKRTLGTEDGGKHIAELHKLGYLPIKIKTIPEGKSVAIKVPMLTIENTHNDFFWLTNYLETLINMSLWQPIVSASVARVYRKTLMSFAEKTCDNQEHIPFQAHDFSMRGMSSLETAETSGAGHLTAFLGTDTIPAISFIEGYYGSKNLIGTSIPATEHSVMSAHGIDELPTFRYLMKKYPNSMLSIVSDTTDFWHNITVNLPILRDEIMARPDHAKIIIRPDSGDSYKIICGDKDAKTEHEQKGLIECLWDTFGGTVNRKGYKVLDCHIGAIYGDGVNYEKMTRILEGLTEKGFASSNLVFGVGSLTYQNHTRDTLGFAVKATSIIINNEEKAIFKNPKTDDGLKKSQKGRVKVLSLDHYIDGLSTKDDFSDDVLETIFENGKLLKEINFDSVRENMLSELNG

SEQ ID NO: 4 - DNA, 1524 bp, Chitinophaga rupis
  source 1..1524: mol_type = genomic DNA
atgcgtatcaatcccattctcttaaaagacggctacaaagtaggccacaaattccaatatcccgaaggtaccagcctggtgtactctaaccttacaccgcgcaaatccaggaacggtgatgtacaggagatcgtgttttttggtttgcagtattttattaaggaatacctgatacgcgagttcaatgaatcttttttcagtcagcctagagaacaggtgctgaaacaatatgcccgccgcatggataattacctgggcaaggatagtattacctacgatcacatagcagccctgcatgacctgggttacctgccactggaaattaaggccctgccggaaggtagcctggtgcccatgcgtgtgccgatctttactattaagaatactataccggaattcttctggctcaccaatatgctggaaactattctcagcgccattctgtggaagccttgtacttctgccaccacggcttttcaatacctgaaaacttttaccaggtatgcaaaagaaaccgtaggtaatgacctgagctttataccctggcaggggcacgacttctctttccgtggtatgagcggtgtggaagatgcgctgatcagcggcgccggtcacctgttatcttttgcaggtacagacactattcccgctattgatttcctggaaacatattataacgcagatgccgaaaaagagctgatcggtggctctgtacctgcaacagaacacagcgtaatgtgtatgggtacgcaggatgatgagatcaaaacctttgaacggctcatcagtgaagtttatcccgcaggcattgtatctattgtaagcgatacctgggatttctggcaggtgatcaccgagtttttacccgcgctgaaaagcaggatcctggcccgtaacggtaaagtagtcatccgtcccgacagcggcgacccggtaaaaattattgtgggcgataaggatgctcccgtaggtagtcccgcttacaaaggcgccattgaatgtatgtgggaaacatttggcggtattattacagagcagggttacaagctgctggatggccacattgggcttatctatggcgatagcatcaccactgaacgccagctggccatactggaagggctgaaacaaaaaggctttgccagctacaacgtagtactgggtattggctcttacacttatgaatatgtaacccgagatacgtttggctttgccatgaaagccacctatggtgaagtgaatggcataggccgggatatatttaaagatcctaaaacagacgacggcaccaagaaatcagccaaaggtttaatgcaggtataccgcaacaccatcaccggtaagctggaagtaaaagaccagtgtacctgggaagaggaagcacagggtgaattgaaaactgtattcaaagatggtaaagtagtggtagactggacactggctgagatcagggaacgtttaaaaggaatgctggaagaaaatgaaaacagtacaacacaaaaagcagtgagcgccggtgtttaa

SEQ ID NO: 5 - protein, 507 aa, Chitinophaga rupis
MRINPILLKDGYKVGHKFQYPEGTSLVYSNLTPRKSRNGDVQEIVFFGLQYFIKEYLIREFNESFFSQPREQVLKQYARRMDNYLGKDSITYDHIAALHDLGYLPLEIKALPEGSLVPMRVPIFTIKNTIPEFFWLTNMLETILSAILWKPCTSATTAFQYLKTFTRYAKETVGNDLSFIPWQGHDFSFRGMSGVEDALISGAGHLLSFAGTDTIPAIDFLETYYNADAEKELIGGSVPATEHSVMCMGTQDDEIKTFERLISEVYPAGIVSIVSDTWDFWQVITEFLPALKSRILARNGKVVIRPDSGDPVKIIVGDKDAPVGSPAYKGAIECMWETFGGIITEQGYKLLDGHIGLIYGDSITTERQLAILEGLKQKGFASYNVVLGIGSYTYEYVTRDTFGFAMKATYGEVNGIGRDIFKDPKTDDGTKKSAKGLMQVYRNTITGKLEVKDQCTWEEEAQGELKTVFKDGKVVVDWTLAEIRERLKGMLEENENSTTQKAVSAGV

SEQ ID NO: 6 - DNA, 1473 bp, Shewanella oneidensis
  source 1..1473: mol_type = genomic DNA
atgtacttgaatcccgttactgctattgatggctacaaagtcgaccaccgtcgtcaatatcccgataatactcaagtgatttttagtaacttgaccgcccgtaaatcccgtcgtggttatacagaccaaatggtattttttggcttgcagtattttatcaagcattacttaattgacagttggaaccgtgatttctttcaacagcccaaagagcaagtgatctgccaattctcccgccgcattaataactatctcggaccgaataatgtcggcactcagcatattgaggagttgcatgatttaggctatttaccaataaaaatcatggcattgcctgaaggctcagtatatccattaaaagtgccttgcttgattttgtacaataccgatgagcggttcttttggttgaccaattatctcgaaaccatcctttccgctaatgtgtggggtatgtgtactagtgctactaccgcgctgcaataccgcaaaatatttgaggcttatgcgttagaaaccgatggtgacatcgcttttgttgattggcagggtcacgattttagtttccgtggcatgtatggtgtagaggccgcgatcatgagcggcgccgcccatttactcagttttactgggacagataccatacccgccattgattttcttgagcaatattaccttgctgatagtgataaagaacttgtcggtggcagtgtgcctgcaacggagcacagcgtgatgtgcgcaggtggcatggagaatgaattagagacgttccgccgtctgattgaagatatttaccctacaggcattgtgagtatcgtttctgattcttgggatttttggcaggtgatgacagaattcaccttagcgttaaaagaccgcattcttgcccgcgatggcaaagtggtgtttaggcctgatacgggttgccctgtgaagatcatttgtggcgatccacaagcaccaatcgggagccctgagtataaaggcgctatcgagtgtttgtgggatgtctttgggggcagcacaactgccaaaggttacaaattacttgatagccatgtcggactgatttatggcgattcaattacgattgaacgggctgaagccatttgtgccggtttgaaggccaaaggttttgcatcaaccaatattgtgtttggaattggcagttttacctatcaacacgtgacccgagatactgacggttatgccgtgaaagcgacctttgcgaaagttgatggtaaagacagagaaatatttaaagatcctaaaactgatgatggcactaaaaaatccgctaagggtttagtagcggtatttaaagatgagcagggtcaattttatcttaaagatcaagccagctggcaagatgttaacaattgcgagtttgtccccgtatttgccgatggtgaattattaacggaatattctttggctgatattcgcgcaagattggcagcgtctcgtcgctga

SEQ ID NO: 7 - protein, 490 aa, Shewanella oneidensis
MYLNPVTAIDGYKVDHRRQYPDNTQVIFSNLTARKSRRGYTDQMVFFGLQYFIKHYLIDSWNRDFFQQPKEQVICQFSRRINNYLGPNNVGTQHIEELHDLGYLPIKIMALPEGSVYPLKVPCLILYNTDERFFWLTNYLETILSANVWGMCTSATTALQYRKIFEAYALETDGDIAFVDWQGHDFSFRGMYGVEAAIMSGAAHLLSFTGTDTIPAIDFLEQYYLADSDKELVGGSVPATEHSVMCAGGMENELETFRRLIEDIYPTGIVSIVSDSWDFWQVMTEFTLALKDRILARDGKVVFRPDTGCPVKIICGDPQAPIGSPEYKGAIECLWDVFGGSTTAKGYKLLDSHVGLIYGDSITIERAEAICAGLKAKGFASTNIVFGIGSFTYQHVTRDTDGYAVKATFAKVDGKDREIFKDPKTDDGTKKSAKGLVAVFKDEQGQFYLKDQASWQDVNNCEFVPVFADGELLTEYSLADIRARLAASRR

SEQ ID NO: 8 - DNA, 1488 bp, Haemophilus ducreyi
  source 1..1488: mol_type = genomic DNA
atggataacctattaaattatagtagtcgtgctagtgctataccatcattattatgcgatttttacaaaacatctcatcgaataatgtatcccgaatgttcacaaattatttatagtacatttacacctcgtagcaatgaacaagcgccttatttaacacaagttgtgtcatttggttttcaagcctttatcattaaatatttaattcattattttaatgataactttttttctcgagataaacatgatgttgtgactgaatactctgcatttattgagaaaaccttacagttagaggatacgggtgaacacattgcaaaattacatgagttgggttatttgcctatccggattaaagctattcctgaaggaaaaacggtggcaattaaagttccggtgatgacgattgaaaatacgcattctgatttcttttggcttactaactatttagaaacattaattaatgtatcactttggcagccgatgacttctgcctcgattgcttttgcttatcggacagcattaattaaatttgctaatgaaacttgtgataatcaagaacatgtgccatttcaatcgcatgatttttcaatgcgtggtatgagttctttagaatccgcagaaacttcaggtgctggccatttaacttcttttttaggtacagacactattcctgcactctcttttgttgaagcgtattatggttcaagcagtctaattggcacgtctatacccgcttctgagcattcagtaatgagttcacatggtgtcgatgaattatcaacatttcgttatttaatggcaaaatttccgcataatatgttgtcaattgtgtcagatactacagacttttggcataacattaccgttaatttgccgttattaaagcaagaaattatagcaaggccagaaaatgcccgtttagtcattcgtccagatagcggtaacttttttgcgattatttgtggtgatccaaccgctgatactgagcatgaacgtaaaggactcattgaatgtttatgggatatttttggtggtacagttaatcagaaaggttataaagtgatcaatccacatattggggcaatttatggtgatggcgtgacttatgaaaaaatgtttaagatcttagaaggattacaagccaaaggatttgcctcaagtaatattgtgtttggcgttggtgcacaaacctatcaacgtaatacacgtgatacgttgggctttgcgcttaaagcgacatctatcactattaatggcgaagaaaaagctattttcaaaaatcctaaaaccgatgatggttttaaaaaatcgcaaaaaggtcgtgttaaagtgctttctcgtgatacttacgttgatggtttaacttcagcggatgattttagtgatgatttattagagctgttatttgaagatggtaagttattacgccaaacagactttgatgaaattcggcaaaacttgttagttagtcgcactacgctatga

SEQ ID NO: 9 - DNA, 1488 bp, Haemophilus ducreyi
  source 1..1488: mol_type = other DNA
atggacaatcttcttaactatagcagccgcgcaagcgccattccgagcctgctgtgtgacttttacaaaacctcgcatcgcatcatgtatcctgaatgctcacagattatttactccacgtttacaccacgctcgaatgaacaagcgccgtatctgacccaggtggtatctttcggtttccaagcgtttatcattaagtacttgatccactattttaacgacaatttcttctcgcgggataaacacgatgtggtaaccgagtattctgctttcatcgagaaaacgctgcagctggaggacactggcgaacacattgcgaagctgcatgaattagggtatctgcccattcggatcaaagccattcccgaagggaaaaccgtagcaatcaaagtgcctgttatgaccatcgagaacacgcattctgacttcttctggttaacgaactacctggaaaccctcattaatgtctctctgtggcagccgatgacgagtgcatcaattgcgttcgcataccgcacggcgctgatcaaatttgccaacgaaacttgcgataaccaggaacatgtgccgttccagtcacacgacttttcgatgcgtggaatgagcagtctggaaagcgctgaaaccagtggagcaggacatttgacgtcctttctgggcaccgatactatcccggctctgtcatttgtggaagcatattatggttcgagtagcctcattgggacttcgattccagcaagcgaacactcagtgatgagctcccacggtgtggatgagctcagcaccttccgttacctgatggctaaatttccgcataacatgttgtctattgtctccgataccaccgacttttggcataacatcacagtcaacttgccgctgctgaaacaagagattattgcccgtccggagaatgcccgtctggttattcgcccagatagtgggaacttctttgcgattatttgtggggatcctacagccgatacggaacatgaacgcaaaggccttatcgaatgcttatgggatatcttcggtggtacagtgaatcagaagggctataaagtcattaacccgcatatcggcgcgatctatggcgatggcgttacctacgaaaagatgttcaaaattctggaaggcttacaagcgaaaggctttgcgagtagcaacattgtctttggtgtaggtgcgcagacatatcaacgcaatactcgcgataccttgggttttgccctgaaagcgacctctattaccatcaatggtgaggagaaagccatctttaagaatccgaaaaccgatgacggcttcaagaaatcgcagaaaggccgcgttaaagtgttgtcccgtgacacttacgttgatggtttaacgagtgctgatgactttagcgacgatctcctcgaactgctgtttgaagatggcaaactgcttcgccaaaccgattttgatgaaattcgtcagaatctgctggtttcccgtacgactttataa

SEQ ID NO: 10 - protein, 495 aa, Haemophilus ducreyi
MDNLLNYSSRASAIPSLLCDFYKTSHRIMYPECSQIIYSTFTPRSNEQAPYLTQVVSFGFQAFIIKYLIHYFNDNFFSRDKHDVVTEYSAFIEKTLQLEDTGEHIAKLHELGYLPIRIKAIPEGKTVAIKVPVMTIENTHSDFFWLTNYLETLINVSLWQPMTSASIAFAYRTALIKFANETCDNQEHVPFQSHDFSMRGMSSLESAETSGAGHLTSFLGTDTIPALSFVEAYYGSSSLIGTSIPASEHSVMSSHGVDELSTFRYLMAKFPHNMLSIVSDTTDFWHNITVNLPLLKQEIIARPENARLVIRPDSGNFFAIICGDPTADTEHERKGLIECLWDIFGGTVNQKGYKVINPHIGAIYGDGVTYEKMFKILEGLQAKGFASSNIVFGVGAQTYQRNTRDTLGFALKATSITINGEEKAIFKNPKTDDGFKKSQKGRVKVLSRDTYVDGLTSADDFSDDLLELLFEDGKLLRQTDFDEIRQNLLVSRTTL

SEQ ID NO: 11 - DNA, 939 bp, Escherichia coli
  source 1..939: mol_type = genomic DNA
atgaagctttttgctggtaacgccaccccggaactagcacaacgtattgccaaccgcctgtacacttcactcggcgacgccgctgtaggtcgctttagcgacggcgaagtcagcgtacaaattaatgaaaatgtacgcggtggtgatattttcatcatccagtccacttgtgcccctactaacgacaacctgatggaattagtcgttatggttgatgccctgcgtcgtgcttccgcaggtcgtatcaccgctgttatcccctactttggctatgcgcgccaggaccgtcgcgtccgttccgctcgtgtaccaatcactgcgaaagtggttgcagacttcctctccagcgtcggtgttgaccgtgtgctgacagtggatctgcacgctgaacagattcagggtttcttcgacgttccggttgataacgtatttggtagcccgatcctgctggaagacatgctgcagctgaatctggataacccaattgtggtttctccggacatcggcggcgttgtgcgtgcccgcgctatcgctaagctgctgaacgataccgatatggcaatcatcgacaaacgtcgtccgcgtgcgaacgtttcacaggtgatgcatatcatcggtgacgttgcaggtcgtgactgcgtactggtcgatgatatgatcgacactggcggtacgctgtgtaaagctgctgaagctctgaaagaacgtggtgctaaacgtgtatttgcgtacgcgactcacccgatcttctctggcaacgcggcgaacaacctgcgtaactctgtaattgatgaagtcgttgtctgcgataccattccgctgagcgatgaaatcaaatcactgccgaacgtgcgtactctgaccctgtcaggtatgctggccgaagcgattcgtcgtatcagcaacgaagaatcgatctctgccatgttcgaacactaa

SEQ ID NO: 12 - protein, 312 aa, Escherichia coli
MKLFAGNATPELAQRIANRLYTSLGDAAVGRFSDGEVSVQINENVRGGDIFIIQSTCAPTNDNLMELVVMVDALRRASAGRITAVIPYFGYARQDRRVRSARVPITAKVVADFLSSVGVDRVLTVDLHAEQIQGFFDVPVDNVFGSPILLEDMLQLNLDNPIVVSPDIGGVVRARAIAKLLNDTDMAIIDKRRPRANVSQVMHIIGDVAGRDCVLVDDMIDTGGTLCKAAEALKERGAKRVFAYATHPIFSGNAANNLRNSVIDEVVVCDTIPLSDEIKSLPNVRTLTLSGMLAEAIRRISNEESISAMFEH

SEQ ID NO: 13 - DNA, 38 bp, synthetic construct
  misc_feature 1..38: note = Forward primer for BhnadV
  source 1..38: mol_type = other DNA
cacaggaaacagaccatgtttaacctgcagcatagcac

SEQ ID NO: 14 - DNA, 40 bp, synthetic construct
  misc_feature 1..40: note = Reverse primer for BhnadV
  source 1..40: mol_type = other DNA
tactgccgccaggcattagccattcagttcactcagcatg

SEQ ID NO: 15 - DNA, 36 bp, synthetic construct
  misc_feature 1..36: note = Forward primer for CrnadV
  source 1..36: mol_type = other DNA
cacaggaaacagaccatgcgtatcaatcccattctc

SEQ ID NO: 16 - DNA, 35 bp, synthetic construct
  misc_feature 1..35: note = Reverse primer for CrnadV
  source 1..35: mol_type = other DNA
tactgccgccaggcattaaacaccggcgctcactg

SEQ ID NO: 17 - DNA, 18 bp, synthetic construct
  misc_feature 1..18: note = Forward primer for pTrc99A
  source 1..18: mol_type = other DNA
tgcctggcggcagtagcg

SEQ ID NO: 18 - DNA, 21 bp, synthetic construct
  misc_feature 1..21: note = Reverse primer for pTrc99A
  source 1..21: mol_type = other DNA
ggtctgtttcctgtgtgaaat

SEQ ID NO: 19 - DNA, 34 bp, synthetic construct
  misc_feature 1..34: note = Forward primer for pTrc99A
  source 1..34: mol_type = other DNA
gcgcgaattgatctggtttgacagcttatcatcg

SEQ ID NO: 20 - DNA, 42 bp, synthetic construct
  misc_feature 1..42: note = Forward primer for prsA
  source 1..42: mol_type = other DNA
tttcacacaggaaacagaccatgaagctttttgctggtaacg

SEQ ID NO: 21 - DNA, 37 bp, synthetic construct
  misc_feature 1..37: note = Reverse primer for prsA
  source 1..37: mol_type = other DNA
gataagctgtcaaacttagtgttcgaacatggcagag

SEQ ID NO: 22 - DNA, 21 bp, synthetic construct
  misc_feature 1..21: note = Forward primer for pBhnadV or pCrnadV
  source 1..21: mol_type = other DNA
gtttgacagcttatcatcgac

SEQ ID NO: 23 - DNA, 21 bp, synthetic construct
  misc_feature 1..21: note = Reverse primer for pBhnadV or pCrnadV
  source 1..21: mol_type = other DNA
cagatcaattcgcgctaactc

SEQ ID NO: 24 - DNA, 38 bp, synthetic construct
  misc_feature 1..38: note = Forward primer for SonadV
  source 1..38: mol_type = other DNA
cacaggaaacagaccatgtacttgaatcccgttactgc

SEQ ID NO: 25 - DNA, 38 bp, synthetic construct
  misc_feature 1..38: note = Reverse primer for SonadV
  source 1..38: mol_type = other DNA
tactgccgccaggcatcagcgacgagacgctgccaatc

SEQ ID NO: 26 - DNA, 41 bp, synthetic construct
  misc_feature 1..41: note = Forward primer for HdnadV
  source 1..41: mol_type = other DNA
cacaggaaacagaccatggacaatcttcttaactatagcag

SEQ ID NO: 27 - DNA, 39 bp, synthetic construct
  misc_feature 1..39: note = Reverse primer for HdnadV
  source 1..39: mol_type = other DNA
tactgccgccaggcattataaagtcgtacgggaaaccag